European Patent Specification EP 3 619 231 B1, published January 28, 2026. Title: Polypeptides. Applicant: Imperial Innovations Ltd. The sequence listing filed with the application follows.

SEQUENCE LISTING (31 sequences)

SEQ ID NO: 1 - protein, 2813 aa, Artificial Sequence
  Synthetic construct
MIPARFAGVLLALALILPGTLCAEGTRGRSSTARCSLFGSDFVNTFDGSMYSFAGYCSYLLAGGCQKRSFSIIGDFQNGKRVSLSVYLGEFFDIHLFVNGTVTQGDQRVSMPYASKGLYLETEAGYYKLSGEAYGFVARIDGSGNFQVLLSDRYFNKTCGLCGNFNIFAEDDFMTQEGTLTSDPYDFANSWALSSGEQWCERASPPSSSCNISSGEMQKGLWEQCQLLKSTSVFARCHPLVDPEPFVALCEKTLCECAGGLECACPALLEYARTCAQEGMVLYGWTDHSACSPVCPAGMEYRQCVSPCARTCQSLHINEMCQERCVDGCSCPEGQLLDEGLCVESTECPCVHSGKRYPPGTSLSRDCNTCICRNSQWICSNEECPGECLVTGQSHFKSFDNRYFTFSGICQYLLARDCQDHSFSIVIETVQCADDRDAVCTRSVTVRLPGLHNSLVKLKHGAGVAMDGQDIQLPLLKGDLRIQHTVTASVRLSYGEDLQMDWDGRGRLLVKLSPVYAGKTCGLCGNYNGNQGDDFLTPSGLAEPRVEDFGNAWKLHGDCQDLQKQHSDPCALNPRMTRFSEEACAVLTSPTFEACHRAVSPLPYLRNCRYDVCSCSDGRECLCGALASYAAACAGRGVRVAWREPGRCELNCPKGQVYLQCGTPCNLTCRSLSYPDEECNEACLEGCFCPPGLYMDERGDCVPKAQCPCYYDGEIFQPEDIFSDHHTMCYCEDGFMHCTMSGVPGSLLPDAVLSSPLSHRSKRSLSCRPPMVKLVCPADNLRAEGLECTKTCQNYDLECMSMGCVSGCLCPPGMVRHENRCVALERCPCFHQGKEYAPGETVKIGCNTCVCRDRKWNCTDHVCDATCSTIGMAHYLTFDGLKYLFPGECQYVLVQDYCGSNPGTFRILVGNKGCSHPSVKCKKRVTILVEGGEIELFDGEVNVKRPMKDETHFEVVESGRYIILLLGKALSVVWDRHLSISVVLKQTYQEKVCGLCGNFDGIQNNDLTSSNLQVEEDPVDFGNSWKVSSQCADTRKVPLDSSPATCHNNIMKQTMVDSSCRILTSDVFQDCNKLVDPEPYLDVCIYDTCSCESIGDCACFCDTIAAYAHVCAQHGKVVTWRTATLCPQSCEERNLRENGYECEWRYNSCAPACQVTCQHPEPLACPVQCVEGCHAHCPPGKILDELLQTCVDPEDCPVCEVAGRRFASGKKVTLNPSDPEHCQICHCDVVNLTCEACQEPGGLVVPPTDAPVSPTTLYVEDISEPPLHDFYCSRLLDLVFLLDGSSRLSEAEFEVLKAFVVDMMERLRISQKWVRVAVVEYHDGSHAYIGLKDRKRPSELRRIASQVKYAGSQVASTSEVLKYTLFQIFSKIDRPEASRIALLLMASQEPQRMSRNFVRYVQGLKKKKVIVIPVGIGPHANLKQIRLIEKQAPENKAFVLSSVDELEQQRDEIVSYLCDLAPEAPPPTLPPHMAQVTVGPGLLGVSTLGPKRNSMVLDVAFVLEGSDKIGEADFNRSKEFMEEVIQRMDVGQDSIHVTVLQYSYMVTVEYPFSEAQSKGDILQRVREIRYQGGNRTNTGLALRYLSDHSFLVSQGDREQAPNLVYMVTGNPASDEIKRLPGDIQVVPIGVGPNANVQELERIGWPNAPILIQDFETLPREAPDLVLQRCCSGEGLQIPTLSPAPDCSQPLDVILLLDGSSSFPASYFDEMKSFAKAFISKANIGPRLTQVSVLQYGSITTIDVPWNVVPEKAHLLSLVDVMQREGGPSQIGDALGFAVRYLTSEMHGARPGASKAVVILVTDVSVDSVDAAADAARSNRVTVFPIGIGDRYDAAQLRILAGPAGDSNVVKLQRIEDLPTMVTLGNSFLHKLCSGFVRICMDEDGNEKRPGDVWTLPDQCHTVTCQPDGQTLLKSHRVNCDRGLRPSCPNSQSPVKVEETCGCRWTCPCVCTGSSTRHIVTFDGQNFKLTGSCSYVLFQNKEQDLEVILHNGACSPGARQGCMKSIEVKHSALSVELHSDMEVTVNGRLVSVPYVGGNMEVNVYGAIMHEVRFNHLGHIFTFTPQNNEFQLQLSPKTFASKTYGLCGICDENGANDFMLRDGTVTTDWKTLVQEWTVQRPGQTCQPILEEQCLVPDSSHCQVLLLPLFAECHKVLAPATFYAICQQDSCHQEQVCEVIASYAHLCRTNGVCVDWRTPDFCAMSCPPSLVYNHCEHGCPRHCDGNVSSCGDHPSEGCFCPPDKVMLEGSCVPEEACTQCIGEDGVQHQFLEAWVPDHQPCQICTCLSGRKVNCTTQPCPTAKAPTCGLCEVARLRQNADQCCPEYECVCDPVSCDLPPVPHCERGLQPTLTNPGECRPNFTCACRKEECKRVSPPSCPPHRLPTLRKTQCCDEYECACNCVNSTVSCPLGYLASTATNDCGCTTTTCLPDKVCVHRSTIYPVGQFWEEGCDVCTCTDMEDAVMGLRVAQCSQKPCEDSCRSGFTYVLHEGECCGRCLPSACEVVTGSPRGDSQSSWKSVGSQWASPENPCLINECVRVKEEVFIQQRNVSCPQLEVPVCPSGFQLSCKTSACCPSCRCERMEACMLNGTVIGPGKTVMIDVCTTCRCMVQVGVISGFKLECRKTTCNPCPLGYKEENNTGECCGRCLPTACTIQLRGGQIMTLKRDETLQDGCDTHFCKVNERGEYFWEKRVTGCPPFDEHKCLAEGGKIMKIPGTCCDTCEEPECNDITARLQYVKVGSCKSEVEVDIHYCQGKCASKAMYSIDINDVQDQCSCCSPTRTEPMQVALHCTNGSVVYHEVLNAMECKCSPRKCSK

SEQ ID NO: 2 - DNA, 8442 bp, Artificial Sequence
  Synthetic construct
atgattcctgccagatttgccggggtgctgcttgctctggccctcattttgccagggaccctttgtgcagaaggaactcgcggcaggtcatccacggcccgatgcagccttttcggaagtgacttcgtcaacacctttgatgggagcatgtacagctttgcgggatactgcagttacctcctggcagggggctgccagaaacgctccttctcgattattggggacttccagaatggcaagagagtgagcctctccgtgtatcttggggaattttttgacatccatttgtttgtcaatggtaccgtgacacagggggaccaaagagtctccatgccctatgcctccaaagggctgtatctagaaactgaggctgggtactacaagctgtccggtgaggcctatggctttgtggccaggatcgatggcagcggcaactttcaagtcctgctgtcagacagatacttcaacaagacctgcgggctgtgtggcaactttaacatctttgctgaagatgactttatgacccaagaagggaccttgacctcggacccttatgactttgccaactcatgggctctgagcagtggagaacagtggtgtgaacgggcatctcctcccagcagctcatgcaacatctcctctggggaaatgcagaagggcctgtgggagcagtgccagcttctgaagagcacctcggtgtttgcccgctgccaccctctggtggaccccgagccttttgtggccctgtgtgagaagactttgtgtgagtgtgctggggggctggagtgcgcctgccctgccctcctggagtacgcccggacctgtgcccaggagggaatggtgctgtacggctggaccgaccacagcgcgtgcagcccagtgtgccctgctggtatggagtataggcagtgtgtgtccccttgcgccaggacctgccagagcctgcacatcaatgaaatgtgtcaggagcgatgcgtggatggctgcagctgccctgagggacagctcctggatgaaggcctctgcgtggagagcaccgagtgtccctgcgtgcattccggaaagcgctaccctcccggcacctccctctctcgagactgcaacacctgcatttgccgaaacagccagtggatctgcagcaatgaagaatgtccaggggagtgccttgtcactggtcaatcccacttcaagagctttgacaacagatacttcaccttcagtgggatctgccagtacctgctggcccgggattgccaggaccactccttctccattgtcattgagactgtccagtgtgctgatgaccgcgacgctgtgtgcacccgctccgtcaccgtccggctgcctggcctgcacaacagccttgtgaaactgaagcatggggcaggagttgccatggatggccaggacatccagctccccctcctgaaaggtgacctccgcatccagcatacagtgacggcctccgtgcgcctcagctacggggaggacctgcagatggactgggatggccgcgggaggctgctggtgaagctgtcccccgtctacgccgggaagacctgcggcctgtgtgggaattacaatggcaaccagggcgacgacttccttaccccctctgggctggcagagccccgggtggaggacttcgggaacgcctggaagctgcacggggactgccaggacctgcagaagcagcacagcgatccctgcgccctcaacccgcgcatgaccaggttctccgaggaggcgtgcgcggtcctgacgtcccccacattcgaggcctgccatcgtgccgtcagcccgctgccctacctgcggaactgccgctacgacgtgtgctcctgctcggacggccgcgagtgcctgtgcggcgccctggccagctatgccgcggcctgcgcggggagaggcgtgcgcgtcgcgtggcgcgagccaggccgctgtgagctgaactgcccgaaaggccaggtgtacctgcagtgcgggaccccctgcaacctgacctgccgctctctctcttacccggatgaggaatgcaatgaggcctgcctggagggctgcttctgccccccagggctctacatggatgagaggggggactgcgtgcccaaggcccagtgcccctgttactatgacggtgagatcttccagccagaagacatcttctcagaccatcacaccatgtgctactgtgaggatggcttcatgcactgtaccatgagtggagtccccggaagcttgctgcctgacgctgtcctcagcagtcccctgtctcatcgcagcaaaaggagcctatcctgtcggccccccatggtcaagctggtgtgtcccgctgacaacctgcgggctgaagggctcgagtgtaccaaaacgtgccagaactatgacctggagtgcatgagcatgggctgtgtctctggctgcctctgccccccgggcatggtccggcatgagaacagatgtgtggccctggaaaggtgtccctgcttccatcagggcaaggagtatgcccctggagaaacagtgaagattggctgcaacacttgtgtctgtcgggaccggaagtggaactgcacagaccatgtgtgtgatgccacgtgctccacgatcggcatggcccactacctcaccttcgacgggctcaaatacctgttccccggggagtgccagtacgttctggtgcaggattactgcggcagtaaccctgggacctttcggatcctagtggggaataagggatgcagccacccctcagtgaaatgcaagaaacgggtcaccatcctggtggagggaggagagattgagctgtttgacggggaggtgaatgtgaagaggcccatgaaggatgagactcactttgaggtggtggagtctggccggtacatcattctgctgctgggcaaagccctctccgtggtctgggaccgccacctgagcatctccgtggtcctgaagcagacataccaggagaaagtgtgtggcctgtgtgggaattttgatggcatccagaacaatgacctcaccagcagcaacctccaagtggaggaagaccctgtggactttgggaactcctggaaagtgagctcgcagtgtgctgacaccagaaaagtgcctctggactcatcccctgccacctgccataacaacatcatgaagcagacgatggtggattcctcctgtagaatccttaccagtgacgtcttccaggactgcaacaagctggtggaccccgagccatatctggatgtctgcatttacgacacctgctcctgtgagtccattggggactgcgcctgcttctgcgacaccattgctgcctatgcccacgtgtgtgcccagcatggcaaggtggtgacctggaggacggccacattgtgcccccagagctgcgaggagaggaatctccgggagaacgggtatgagtgtgagtggcgctataacagctgtgcacctgcctgtcaagtcacgtgtcagcaccctgagccactggcctgccctgtgcagtgtgtggagggctgccatgcccactgccctccagggaaaatcctggatgagcttttgcagacctgcgttgaccctgaagactgtccagtgtgtgaggtggctggccggcgttttgcctcaggaaagaaagtcaccttgaatcccagtgaccctgagcactgccagatttgccactgtgatgttgtcaacctcacctgtgaagcctgccaggagccgggaggcctggtggtgcctcccacagatgccccggtgagccccaccactctgtatgtggaggacatctcggaaccgccgttgcacgatttctactgcagcaggctactggacctggtcttcctgctggatggctcctccaggctgtccgaggctgagtttgaagtgctgaaggcctttgtggtggacatgatggagcggctgcgcatctcccagaagtgggtccgcgtggccgtggtggagtaccacgacggctcccacgcctacatcgggctcaaggaccggaagcgaccgtcagagctgcggcgcattgccagccaggtgaagtatgcgggcagccaggtggcctccaccagcgaggtcttgaaatacacactgttccaaatcttcagcaagatcgaccgccctgaagcctcccgcatcgccctgctcctgatggccagccaggagccccaacggatgtcccggaactttgtccgctacgtccagggcctgaagaagaagaaggtcattgtgatcccggtgggcattgggccccatgccaacctcaagcagatccgcctcatcgagaagcaggcccctgagaacaaggccttcgtgctgagcagtgtggatgagctggagcagcaaagggacgagatcgttagctacctctgtgaccttgcccctgaagcccctcctcctactctgcccccccacatggcacaagtcactgtgggcccggggctcttgggggtttcgaccctggggcccaagaggaactccatggttctggatgtggcgttcgtcctggaaggatcggacaaaattggtgaagccgacttcaacaggagcaaggagttcatggaggaggtgattcagcggatggatgtgggccaggacagcatccacgtcacggtgctgcagtactcctacatggtgaccgtggagtaccccttcagcgaggcacagtccaaaggggacatcctgcagcgggtgcgagagatccgctaccagggcggcaacaggaccaacactgggctggccctgcggtacctctctgaccacagcttcttggtcagccagggtgaccgggagcaggcgcccaacctggtctacatggtcaccggaaatcctgcctctgatgagatcaagaggctgcctggagacatccaggtggtgcccattggagtgggccctaatgccaacgtgcaggagctggagaggattggctggcccaatgcccctatcctcatccaggactttgagacgctcccccgagaggctcctgacctggtgctgcagaggtgctgctccggagaggggctgcagatccccaccctctcccctgcacctgactgcagccagcccctggacgtgatccttctcctggatggctcctccagtttcccagcttcttattttgatgaaatgaagagtttcgccaaggctttcatttcaaaagccaatatagggcctcgtctcactcaggtgtcagtgctgcagtatggaagcatcaccaccattgacgtgccatggaacgtggtcccggagaaagcccatttgctgagccttgtggacgtcatgcagcgggagggaggccccagccaaatcggggatgccttgggctttgctgtgcgatacttgacttcagaaatgcatggtgccaggccgggagcctcaaaggcggtggtcatcctggtcacggacgtctctgtggattcagtggatgcagcagctgatgccgccaggtccaacagagtgacagtgttccctattggaattggagatcgctacgatgcagcccagctacggatcttggcaggcccagcaggcgactccaacgtggtgaagctccagcgaatcgaagacctccctaccatggtcaccttgggcaattccttcctccacaaactgtgctctggatttgttaggatttgcatggatgaggatgggaatgagaagaggcccggggacgtctggaccttgccagaccagtgccacaccgtgacttgccagccagatggccagaccttgctgaagagtcatcgggtcaactgtgaccgggggctgaggccttcgtgccctaacagccagtcccctgttaaagtggaagagacctgtggctgccgctggacctgcccctgcgtgtgcacaggcagctccactcggcacatcgtgacctttgatgggcagaatttcaagctgactggcagctgttcttatgtcctatttcaaaacaaggagcaggacctggaggtgattctccataatggtgcctgcagccctggagcaaggcagggctgcatgaaatccatcgaggtgaagcacagtgccctctccgtcgagctgcacagtgacatggaggtgacggtgaatgggagactggtctctgttccttacgtgggtgggaacatggaagtcaacgtttatggtgccatcatgcatgaggtcagattcaatcaccttggtcacatcttcacattcactccacaaaacaatgagttccaactgcagctcagccccaagacttttgcttcaaagacgtatggtctgtgtgggatctgtgatgagaacggagccaatgacttcatgctgagggatggcacagtcaccacagactggaaaacacttgttcaggaatggactgtgcagcggccagggcagacgtgccagcccatcctggaggagcagtgtcttgtccccgacagctcccactgccaggtcctcctcttaccactgtttgctgaatgccacaaggtcctggctccagccacattctatgccatctgccagcaggacagttgccaccaggagcaagtgtgtgaggtgatcgcctcttatgcccacctctgtcggaccaacggggtctgcgttgactggaggacacctgatttctgtgctatgtcatgcccaccatctctggtctacaaccactgtgagcatggctgtccccggcactgtgatggcaacgtgagctcctgtggggaccatccctccgaaggctgtttctgccctccagataaagtcatgttggaaggcagctgtgtccctgaagaggcctgcactcagtgcattggtgaggatggagtccagcaccagttcctggaagcctgggtcccggaccaccagccctgtcagatctgcacatgcctcagcgggcggaaggtcaactgcacaacgcagccctgccccacggccaaagctcccacgtgtggcctgtgtgaagtagcccgcctccgccagaatgcagaccagtgctgccccgagtatgagtgtgtgtgtgacccagtgagctgtgacctgcccccagtgcctcactgtgaacgtggcctccagcccacactgaccaaccctggcgagtgcagacccaacttcacctgcgcctgcaggaaggaggagtgcaaaagagtgtccccaccctcctgccccccgcaccgtttgcccacccttcggaagacccagtgctgtgatgagtatgagtgtgcctgcaactgtgtcaactccacagtgagctgtccccttgggtacttggcctcaaccgccaccaatgactgtggctgtaccacaaccacctgccttcccgacaaggtgtgtgtccaccgaagcaccatctaccctgtgggccagttctgggaggagggctgcgatgtgtgcacctgcaccgacatggaggatgccgtgatgggcctccgcgtggcccagtgctcccagaagccctgtgaggacagctgtcggtcgggcttcacttacgttctgcatgaaggcgagtgctgtggaaggtgcctgccatctgcctgtgaggtggtgactggctcaccgcggggggactcccagtcttcctggaagagtgtcggctcccagtgggcctccccggagaacccctgcctcatcaatgagtgtgtccgagtgaaggaggaggtctttatacaacaaaggaacgtctcctgcccccagctggaggtccctgtctgcccctcgggctttcagctgagctgtaagacctcagcgtgctgcccaagctgtcgctgtgagcgcatggaggcctgcatgctcaatggcactgtcattgggcccgggaagactgtgatgatcgatgtgtgcacgacctgccgctgcatggtgcaggtgggggtcatctctggattcaagctggagtgcaggaagaccacctgcaacccctgccccctgggttacaaggaagaaaataacacaggtgaatgttgtgggagatgtttgcctacggcttgcaccattcagctaagaggaggacagatcatgacactgaagcgtgatgagacgctccaggatggctgtgatactcacttctgcaaggtcaatgagagaggagagtacttctgggagaagagggtcacaggctgcccaccctttgatgaacacaagtgtctggctgagggaggtaaaattatgaaaattccaggcacctgctgtgacacatgtgaggagcctgagtgcaacgacatcactgccaggctgcagtatgtcaaggtgggaagctgtaagtctgaagtagaggtggatatccactactgccagggcaaatgtgccagcaaagccatgtactccattgacatcaacgatgtgcaggaccagtgctcctgctgctctccgacacggacggagcccatgcaggtggccctgcactgcaccaatggctctgttgtgtaccatgaggttctcaatgccatggagtgcaaatgctcccccaggaagtgcagcaagtga

SEQ ID NO: 3 - protein, 1967 aa, Artificial Sequence
  Synthetic construct
MIPARFAGVLLALALILPGTLCAEGTRGRSSTARCSLFGSDFVNTFDGSMYSFAGYCSYLLAGGCQKRSFSIIGDFQNGKRVSLSVYLGEFFDIHLFVNGTVTQGDQRVSMPYASKGLYLETEAGYYKLSGEAYGFVARIDGSGNFQVLLSDRYFNKTCGLCGNFNIFAEDDFMTQEGTLTSDPYDFANSWALSSGEQWCERASPPSSSCNISSGEMQKGLWEQCQLLKSTSVFARCHPLVDPEPFVALCEKTLCECAGGLECACPALLEYARTCAQEGMVLYGWTDHSACSPVCPAGMEYRQCVSPCARTCQSLHINEMCQERCVDGCSCPEGQLLDEGLCVESTECPCVHSGKRYPPGTSLSRDCNTCICRNSQWICSNEECPGECLVTGQSHFKSFDNRYFTFSGICQYLLARDCQDHSFSIVIETVQCADDRDAVCTRSVTVRLPGLHNSLVKLKHGAGVAMDGQDIQLPLLKGDLRIQHTVTASVRLSYGEDLQMDWDGRGRLLVKLSPVYAGKTCGLCGNYNGNQGDDFLTPSGLAEPRVEDFGNAWKLHGDCQDLQKQHSDPCALNPRMTRFSEEACAVLTSPTFEACHRAVSPLPYLRNCRYDVCSCSDGRECLCGALASYAAACAGRGVRVAWREPGRCELNCPKGQVYLQCGTPCNLTCRSLSYPDEECNEACLEGCFCPPGLYMDERGDCVPKAQCPCYYDGEIFQPEDIFSDHHTMCYCEDGFMHCTMSGVPGSLLPDAVLSSPLSHRSKRSLSCRPPMVKLVCPADNLRAEGLECTKTCQNYDLECMSMGCVSGCLCPPGMVRHENRCVALERCPCFHQGKEYAPGETVKIGCNTCVCRDRKWNCTDHVCDATCSTIGMAHYLTFDGLKYLFPGECQYVLVQDYCGSNPGTFRILVGNKGCSHPSVKCKKRVTILVEGGEIELFDGEVNVKRPMKDETHFEVVESGRYIILLLGKALSVVWDRHLSISVVLKQTYQEKVCGLCGNFDGIQNNDLTSSNLQVEEDPVDFGNSWKVSSQCADTRKVPLDSSPATCHNNIMKQTMVDSSCRILTSDVFQDCNKLVDPEPYLDVCIYDTCSCESIGDCACFCDTIAAYAHVCAQHGKVVTWRTATLCPQSCEERNLRENGYECEWRYNSCAPACQVTCQHPEPLACPVQCVEGCHAHCPPGKILDELLQTCVDPEDCPVCEVAGRRFASGKKVTLNPSDPEHCQICHCDVVNLTCEACQEPGGLVVPPTDAPVSPTTLYVEDISEPPLHDFYCSRLLDLVFLLDGSSRLSEAEFEVLKAFVVDMMERLRISQKWVRVAVVEYHDGSHAYIGLKDRKRPSELRRIASQVKYAGSQVASTSEVLKYTLFQIFSKIDRPEASRIALLLMASQEPQRMSRNFVRYVQGLKKKKVIVIPVGIGPHANLKQIRLIEKQAPENKAFVLSSVDELEQQRDEIVSYLCDLAPEAPPPTLPPHMAQVTVGPGLLGVSTLGPKRNSMVLDVAFVLEGSDKIGEADFNRSKEFMEEVIQRMDVGQDSIHVTVLQYSYMVTVEYPFSEAQSKGDILQRVREIRYQGGNRTNTGLALRYLSDHSFLVSQGDREQAPNLVYMVTGNPASDEIKRLPGDIQVVPIGVGPNANVQELERIGWPNAPILIQDFETLPREAPDLVLQRCCSGEGLQIPTLSPAPDCSQPLDVILLLDGSSSFPASYFDEMKSFAKAFISKANIGPRLTQVSVLQYGSITTIDVPWNVVPEKAHLLSLVDVMQREGGPSQIGDALGFAVRYLTSEMHGARPGASKAVVILVTDVSVDSVDAAADAARSNRVTVFPIGIGDRYDAAQLRILAGPAGDSNVVKLQRIEDLPTMVTLGNSFLHKLCSGEPECNDITARLQYVKVGSCKSEVEVDIHYCQGKCASKAMYSIDINDVQDQCSCCSPTRTEPMQVALHCTNGSVVYHEVLNAMECKCSPRKCSK

SEQ ID NO: 4 - DNA, 5904 bp, Artificial Sequence
  Synthetic construct
atgattcctgccagatttgccggggtgctgcttgctctggccctcattttgccagggaccctttgtgcagaaggaactcgcggcaggtcatccacggcccgatgcagccttttcggaagtgacttcgtcaacacctttgatgggagcatgtacagctttgcgggatactgcagttacctcctggcagggggctgccagaaacgctccttctcgattattggggacttccagaatggcaagagagtgagcctctccgtgtatcttggggaattttttgacatccatttgtttgtcaatggtacggtgacacagggggaccaaagagtctccatgccctatgcctccaaagggctgtatctagaaactgaggctgggtactacaagctgtccggtgaggcctatggctttgtggccaggatcgatggcagcggcaactttcaagtcctgctgtcagacagatacttcaacaagacctgcgggctgtgtggcaactttaacatctttgctgaagatgactttatgacccaagaagggaccttgacctcggacccttatgactttgccaactcatgggctctgagcagtggagaacagtggtgtgaacgggcatctcctcccagcagctcatgcaacatctcctctggggaaatgcagaagggcctgtgggagcagtgccagcttctgaagagcacctcggtgtttgcccgctgccaccctctggtggaccccgagccttttgtggccctgtgtgagaagactttgtgtgagtgtgctggggggctggagtgcgcctgccctgccctcctggagtacgcccggacctgtgcccaggagggaatggtgctgtacggctggaccgaccacagcgcgtgcagcccagtgtgccctgctggtatggagtataggcagtgtgtgtccccttgcgccaggacctgccagagcctgcacatcaatgaaatgtgtcaggagcgatgcgtggatggctgcagctgccctgagggacagctcctggatgaaggcctctgcgtggagagcaccgagtgtccctgcgtgcattccggaaagcgctaccctcccggcacctccctctctcgagactgcaacacctgcatttgccgaaacagccagtggatctgcagcaatgaagaatgtccaggggagtgccttgtcactggtcaatcccacttcaagagctttgacaacagatacttcaccttcagtgggatctgccagtacctgctggcccgggattgccaggaccactccttctccattgtcattgagactgtccagtgtgctgatgaccgcgacgctgtgtgcacccgctccgtcaccgtccggctgcctggcctgcacaacagccttgtgaaactgaagcatggggcaggagttgccatggatggccaggacatccagctccccctcctgaaaggtgacctccgcatccagcatacagtgacggcctccgtgcgcctcagctacggggaggacctgcagatggactgggatggccgcgggaggctgctggtgaagctgtcccccgtctacgccgggaagacctgcggcctgtgtgggaattacaatggcaaccagggcgacgacttccttaccccctctgggctggcagagccccgggtggaggacttcgggaacgcctggaagctgcacggggactgccaggacctgcagaagcagcacagcgatccctgcgccctcaacccgcgcatgaccaggttctccgaggaggcgtgcgcggtcctgacgtcccccacattcgaggcctgccatcgtgccgtcagcccgctgccctacctgcggaactgccgctacgacgtgtgctcctgctcggacggccgcgagtgcctgtgcggcgccctggccagctatgccgcggcctgcgcggggagaggcgtgcgcgtcgcgtggcgcgagccaggccgctgtgagctgaactgcccgaaaggccaggtgtacctgcagtgcgggaccccctgcaacctgacctgccgctctctctcttacccggatgaggaatgcaatgaggcctgcctggagggctgcttctgccccccagggctctacatggatgagaggggggactgcgtgcccaaggcccagtgcccctgttactatgacggtgagatcttccagccagaagacatcttctcagaccatcacaccatgtgctactgtgaggatggcttcatgcactgtaccatgagtggagtccccggaagcttgctgcctgacgctgtcctcagcagtcccctgtctcatcgcagcaaaaggagcctatcctgtcggccccccatggtcaagctggtgtgtcccgctgacaacctgcgggctgaagggctcgagtgtaccaaaacgtgccagaactatgacctggagtgcatgagcatgggctgtgtctctggctgcctctgccccccgggcatggtccggcatgagaacagatgtgtggccctggaaaggtgtccctgcttccatcagggcaaggagtatgcccctggagaaacagtgaagattggctgcaacacttgtgtctgtcgggaccggaagtggaactgcacagaccatgtgtgtgatgccacgtgctccacgatcggcatggcccactacctcaccttcgacgggctcaaatacctgttccccggggagtgccagtacgttctggtgcaggattactgcggcagtaaccctgggacctttcggatcctagtggggaataagggatgcagccacccctcagtgaaatgcaagaaacgggtcaccatcctggtggagggaggagagattgagctgtttgacggggaggtgaatgtgaagaggcccatgaaggatgagactcactttgaggtggtggagtctggccggtacatcattctgctgctgggcaaagccctctccgtggtctgggaccgccacctgagcatctccgtggtcctgaagcagacataccaggagaaagtgtgtggcctgtgtgggaattttgatggcatccagaacaatgacctcaccagcagcaacctccaagtggaggaagaccctgtggactttgggaactcctggaaagtgagctcgcagtgtgctgacaccagaaaagtgcctctggactcatcccctgccacctgccataacaacatcatgaagcagacgatggtggattcctcctgtagaatccttaccagtgacgtcttccaggactgcaacaagctggtggaccccgagccatatctggatgtctgcatttacgacacctgctcctgtgagtccattggggactgcgcctgcttctgcgacaccattgctgcctatgcccacgtgtgtgcccagcatggcaaggtggtgacctggaggacggccacattgtgcccccagagctgcgaggagaggaatctccgggagaacgggtatgagtgtgagtggcgctataacagctgtgcacctgcctgtcaagtcacgtgtcagcaccctgagccactggcctgccctgtgcagtgtgtggagggctgccatgcccactgccctccagggaaaatcctggatgagcttttgcagacctgcgttgaccctgaagactgtccagtgtgtgaggtggctggccggcgttttgcctcaggaaagaaagtcaccttgaatcccagtgaccctgagcactgccagatttgccactgtgatgttgtcaacctcacctgtgaagcctgccaggagccgggaggcctggtggtgcctcccacagatgccccggtgagccccaccactctgtatgtggaggacatctcggaaccgccgttgcacgatttctactgcagcaggctactggacctggtcttcctgctggatggctcctccaggctgtccgaggctgagtttgaagtgctgaaggcctttgtggtggacatgatggagcggctgcgcatctcccagaagtgggtccgcgtggccgtggtggagtaccacgacggctcccacgcctacatcgggctcaaggaccggaagcgaccgtcagagctgcggcgcattgccagccaggtgaagtatgcgggcagccaggtggcctccaccagcgaggtcttgaaatacacactgttccaaatcttcagcaagatcgaccgccctgaagcctcccgcatcgccctgctcctgatggccagccaggagccccaacggatgtcccggaactttgtccgctacgtccagggcctgaagaagaagaaggtcattgtgatcccggtgggcattgggccccatgccaacctcaagcagatccgcctcatcgagaagcaggcccctgagaacaaggccttcgtgctgagcagtgtggatgagctggagcagcaaagggacgagatcgttagctacctctgtgaccttgcccctgaagcccctcctcctactctgcccccccacatggcacaagtcactgtgggcccggggctcttgggggtttcgaccctggggcccaagaggaactccatggttctggatgtggcgttcgtcctggaaggatcggacaaaattggtgaagccgacttcaacaggagcaaggagttcatggaggaggtgattcagcggatggatgtgggccaggacagcatccacgtcacggtgctgcagtactcctacatggtgaccgtggagtaccccttcagcgaggcacagtccaaaggggacatcctgcagcgggtgcgagagatccgctaccagggcggcaacaggaccaacactgggctggccctgcggtacctctctgaccacagcttcttggtcagccagggtgaccgggagcaggcgcccaacctggtctacatggtcaccggaaatcctgcctctgatgagatcaagaggctgcctggagacatccaggtggtgcccattggagtgggccctaatgccaacgtgcaggagctggagaggattggctggcccaatgcccctatcctcatccaggactttgagacgctcccccgagaggctcctgacctggtgctgcagaggtgctgctccggagaggggctgcagatccccaccctctcccctgcacctgactgcagccagcccctggacgtgatccttctcctggatggctcctccagtttcccagcttcttattttgatgaaatgaagagtttcgccaaggctttcatttcaaaagccaatatagggcctcgtctcactcaggtgtcagtgctgcagtatggaagcatcaccaccattgacgtgccatggaacgtggtcccggagaaagcccatttgctgagccttgtggacgtcatgcagcgggagggaggccccagccaaatcggggatgccttgggctttgctgtgcgatacttgacttcagaaatgcatggtgccaggccgggagcctcaaaggcggtggtcatcctggtcacggacgtctctgtggattcagtggatgcagcagctgatgccgccaggtccaacagagtgacagtgttccctattggaattggagatcgctacgatgcagcccagctacggatcttggcaggcccagcaggcgactccaacgtggtgaagctccagcgaatcgaagacctccctaccatggtcaccttgggcaattccttcctccacaaactgtgctctggagagcctgagtgcaacgacatcactgccaggctgcagtatgtcaaggtgggaagctgtaagtctgaagtagaggtggatatccactactgccagggcaaatgtgccagcaaagccatgtactccattgacatcaacgatgtgcaggaccagtgctcctgctgctctccgacacggacggagcccatgcaggtggccctgcactgcaccaatggctctgttgtgtaccatgaggttctcaatgccatggagtgcaaatgctcccccaggaagtgcagcaagtga

SEQ ID NO: 5 - protein, 22 aa, Artificial Sequence
  Synthetic construct
MIPARFAGVLLALALILPGTLC

SEQ ID NO: 6 - protein, 741 aa, Artificial Sequence
  Synthetic construct
AEGTRGRSSTARCSLFGSDFVNTFDGSMYSFAGYCSYLLAGGCQKRSFSIIGDFQNGKRVSLSVYLGEFFDIHLFVNGTVTQGDQRVSMPYASKGLYLETEAGYYKLSGEAYGFVARIDGSGNFQVLLSDRYFNKTCGLCGNFNIFAEDDFMTQEGTLTSDPYDFANSWALSSGEQWCERASPPSSSCNISSGEMQKGLWEQCQLLKSTSVFARCHPLVDPEPFVALCEKTLCECAGGLECACPALLEYARTCAQEGMVLYGWTDHSACSPVCPAGMEYRQCVSPCARTCQSLHINEMCQERCVDGCSCPEGQLLDEGLCVESTECPCVHSGKRYPPGTSLSRDCNTCICRNSQWICSNEECPGECLVTGQSHFKSFDNRYFTFSGICQYLLARDCQDHSFSIVIETVQCADDRDAVCTRSVTVRLPGLHNSLVKLKHGAGVAMDGQDIQLPLLKGDLRIQHTVTASVRLSYGEDLQMDWDGRGRLLVKLSPVYAGKTCGLCGNYNGNQGDDFLTPSGLAEPRVEDFGNAWKLHGDCQDLQKQHSDPCALNPRMTRFSEEACAVLTSPTFEACHRAVSPLPYLRNCRYDVCSCSDGRECLCGALASYAAACAGRGVRVAWREPGRCELNCPKGQVYLQCGTPCNLTCRSLSYPDEECNEACLEGCFCPPGLYMDERGDCVPKAQCPCYYDGEIFQPEDIFSDHHTMCYCEDGFMHCTMSGVPGSLLPDAVLSSPLSHRSKR

SEQ ID NO: 7 - protein, 101 aa, Artificial Sequence
  Synthetic construct
SLSCRPPMVKLVCPADNLRAEGLECTKTCQNYDLECMSMGCVSGCLCPPGMVRHENRCVALERCPCFHQGKEYAPGETVKIGCNTCVCRDRKWNCTDHVCD

SEQ ID NO: 8 - protein, 406 aa, Artificial Sequence
  Synthetic construct
ATCSTIGMAHYLTFDGLKYLFPGECQYVLVQDYCGSNPGTFRILVGNKGCSHPSVKCKKRVTILVEGGEIELFDGEVNVKRPMKDETHFEVVESGRYIILLLGKALSVVWDRHLSISVVLKQTYQEKVCGLCGNFDGIQNNDLTSSNLQVEEDPVDFGNSWKVSSQCADTRKVPLDSSPATCHNNIMKQTMVDSSCRILTSDVFQDCNKLVDPEPYLDVCIYDTCSCESIGDCACFCDTIAAYAHVCAQHGKVVTWRTATLCPQSCEERNLRENGYECEWRYNSCAPACQVTCQHPEPLACPVQCVEGCHAHCPPGKILDELLQTCVDPEDCPVCEVAGRRFASGKKVTLNPSDPEHCQICHCDVVNLTCEACQEPGGLVVPPTDAPVSPTTLYVEDISEPPLHDF

SEQ ID NO: 9 - protein, 183 aa, Artificial Sequence
  Synthetic construct
YCSRLLDLVFLLDGSSRLSEAEFEVLKAFVVDMMERLRISQKWVRVAVVEYHDGSHAYIGLKDRKRPSELRRIASQVKYAGSQVASTSEVLKYTLFQIFSKIDRPEASRIALLLMASQEPQRMSRNFVRYVQGLKKKKVIVIPVGIGPHANLKQIRLIEKQAPENKAFVLSSVDELEQQRDEI

SEQ ID NO: 10 - protein, 44 aa, Artificial Sequence
  Synthetic construct
VSYLCDLAPEAPPPTLPPHMAQVTVGPGLLGVSTLGPKRNSMVL

SEQ ID NO: 11 - protein, 173 aa, Artificial Sequence
  Synthetic construct
DVAFVLEGSDKIGEADFNRSKEFMEEVIQRMDVGQDSIHVTVLQYSYMVTVEYPFSEAQSKGDILQRVREIRYQGGNRTNTGLALRYLSDHSFLVSQGDREQAPNLVYMVTGNPASDEIKRLPGDIQVVPIGVGPNANVQELERIGWPNAPILIQDFETLPREAPDLVLQRCC

SEQ ID NO: 12 - protein, 204 aa, Artificial Sequence
  Synthetic construct
SGEGLQIPTLSPAPDCSQPLDVILLLDGSSSFPASYFDEMKSFAKAFISKANIGPRLTQVSVLQYGSITTIDVPWNVVPEKAHLLSLVDVMQREGGPSQIGDALGFAVRYLTSEMHGARPGASKAVVILVTDVSVDSVDAAADAARSNRVTVFPIGIGDRYDAAQLRILAGPAGDSNVVKLQRIEDLPTMVTLGNSFLHKLCSG

SEQ ID NO: 13 - protein, 380 aa, Artificial Sequence
  Synthetic construct
FVRICMDEDGNEKRPGDVWTLPDQCHTVTCQPDGQTLLKSHRVNCDRGLRPSCPNSQSPVKVEETCGCRWTCPCVCTGSSTRHIVTFDGQNFKLTGSCSYVLFQNKEQDLEVILHNGACSPGARQGCMKSIEVKHSALSVELHSDMEVTVNGRLVSVPYVGGNMEVNVYGAIMHEVRFNHLGHIFTFTPQNNEFQLQLSPKTFASKTYGLCGICDENGANDFMLRDGTVTTDWKTLVQEWTVQRPGQTCQPILEEQCLVPDSSHCQVLLLPLFAECHKVLAPATFYAICQQDSCHQEQVCEVIASYAHLCRTNGVCVDWRTPDFCAMSCPPSLVYNHCEHGCPRHCDGNVSSCGDHPSEGCFCPPDKVMLEGSCVPEEAC

SEQ ID NO: 14 - protein, 79 aa, Artificial Sequence
  Synthetic construct
TQCIGEDGVQHQFLEAWVPDHQPCQICTCLSGRKVNCTTQPCPTAKAPTCGLCEVARLRQNADQCCPEYECVCDPVSCD

SEQ ID NO: 15 - protein, 69 aa, Artificial Sequence
  Synthetic construct
LPPVPHCERGLQPTLTNPGECRPNFTCACRKEECKRVSPPSCPPHRLPTLRKTQCCDEYECACNCVNST

SEQ ID NO: 16 - protein, 26 aa, Artificial Sequence
  Synthetic construct
VSCPLGYLASTATNDCGCTTTTCLPD

SEQ ID NO: 17 - protein, 68 aa, Artificial Sequence
  Synthetic construct
KVCVHRSTIYPVGQFWEEGCDVCTCTDMEDAVMGLRVAQCSQKPCEDSCRSGFTYVLHEGECCGRCLP

SEQ ID NO: 18 - protein, 81 aa, Artificial Sequence
  Synthetic construct
SACEVVTGSPRGDSQSSWKSVGSQWASPENPCLINECVRVKEEVFIQQRNVSCPQLEVPVCPSGFQLSCKTSACCPSCRCE

SEQ ID NO: 19 - protein, 69 aa, Artificial Sequence
  Synthetic construct
RMEACMLNGTVIGPGKTVMIDVCTTCRCMVQVGVISGFKLECRKTTCNPCPLGYKEENNTGECCGRCLP

SEQ ID NO: 20 - protein, 74 aa, Artificial Sequence
  Synthetic construct
TACTIQLRGGQIMTLKRDETLQDGCDTHFCKVNERGEYFWEKRVTGCPPFDEHKCLAEGGKIMKIPGTCCDTCE

SEQ ID NO: 21 - protein, 93 aa, Artificial Sequence
  Synthetic construct
EPECNDITARLQYVKVGSCKSEVEVDIHYCQGKCASKAMYSIDINDVQDQCSCCSPTRTEPMQVALHCTNGSVVYHEVLNAMECKCSPRKCSK

SEQ ID NO: 22 - DNA, 2538 bp, Artificial Sequence
  Synthetic construct
tttgttaggatttgcatggatgaggatgggaatgagaagaggcccggggacgtctggaccttgccagaccagtgccacaccgtgacttgccagccagatggccagaccttgctgaagagtcatcgggtcaactgtgaccgggggctgaggccttcgtgccctaacagccagtcccctgttaaagtggaagagacctgtggctgccgctggacctgcccctgcgtgtgcacaggcagctccactcggcacatcgtgacctttgatgggcagaatttcaagctgactggcagctgttcttatgtcctatttcaaaacaaggagcaggacctggaggtgattctccataatggtgcctgcagccctggagcaaggcagggctgcatgaaatccatcgaggtgaagcacagtgccctctccgtcgagctgcacagtgacatggaggtgacggtgaatgggagactggtctctgttccttacgtgggtgggaacatggaagtcaacgtttatggtgccatcatgcatgaggtcagattcaatcaccttggtcacatcttcacattcactccacaaaacaatgagttccaactgcagctcagccccaagacttttgcttcaaagacgtatggtctgtgtgggatctgtgatgagaacggagccaatgacttcatgctgagggatggcacagtcaccacagactggaaaacacttgttcaggaatggactgtgcagcggccagggcagacgtgccagcccatcctggaggagcagtgtcttgtccccgacagctcccactgccaggtcctcctcttaccactgtttgctgaatgccacaaggtcctggctccagccacattctatgccatctgccagcaggacagttgccaccaggagcaagtgtgtgaggtgatcgcctcttatgcccacctctgtcggaccaacggggtctgcgttgactggaggacacctgatttctgtgctatgtcatgcccaccatctctggtctacaaccactgtgagcatggctgtccccggcactgtgatggcaacgtgagctcctgtggggaccatccctccgaaggctgtttctgccctccagataaagtcatgttggaaggcagctgtgtccctgaagaggcctgcactcagtgcattggtgaggatggagtccagcaccagttcctggaagcctgggtcccggaccaccagccctgtcagatctgcacatgcctcagcgggcggaaggtcaactgcacaacgcagccctgccccacggccaaagctcccacgtgtggcctgtgtgaagtagcccgcctccgccagaatgcagaccagtgctgccccgagtatgagtgtgtgtgtgacccagtgagctgtgacctgcccccagtgcctcactgtgaacgtggcctccagcccacactgaccaaccctggcgagtgcagacccaacttcacctgcgcctgcaggaaggaggagtgcaaaagagtgtccccaccctcctgccccccgcaccgtttgcccacccttcggaagacccagtgctgtgatgagtatgagtgtgcctgcaactgtgtcaactccacagtgagctgtccccttgggtacttggcctcaaccgccaccaatgactgtggctgtaccacaaccacctgccttcccgacaaggtgtgtgtccaccgaagcaccatctaccctgtgggccagttctgggaggagggctgcgatgtgtgcacctgcaccgacatggaggatgccgtgatgggcctccgcgtggcccagtgctcccagaagccctgtgaggacagctgtcggtcgggcttcacttacgttctgcatgaaggcgagtgctgtggaaggtgcctgccatctgcctgtgaggtggtgactggctcaccgcggggggactcccagtcttcctggaagagtgtcggctcccagtgggcctccccggagaacccctgcctcatcaatgagtgtgtccgagtgaaggaggaggtctttatacaacaaaggaacgtctcctgcccccagctggaggtccctgtctgcccctcgggctttcagctgagctgtaagacctcagcgtgctgcccaagctgtcgctgtgagcgcatggaggcctgcatgctcaatggcactgtcattgggcccgggaagactgtgatgatcgatgtgtgcacgacctgccgctgcatggtgcaggtgggggtcatctctggattcaagctggagtgcaggaagaccacctgcaacccctgccccctgggttacaaggaagaaaataacacaggtgaatgttgtgggagatgtttgcctacggcttgcaccattcagctaagaggaggacagatcatgacactgaagcgtgatgagacgctccaggatggctgtgatactcacttctgcaaggtcaatgagagaggagagtacttctgggagaagagggtcacaggctgcccaccctttgatgaacacaagtgtctggctgagggaggtaaaattatgaaaattccaggcacctgctgtgacacatgtgag

SEQ ID NO: 23 - protein, 22 aa, Artificial Sequence
  Synthetic construct
MIPARFAGVLLALALILPGTLC

SEQ ID NO: 24 - protein, 741 aa, Artificial Sequence; identical to SEQ ID NO: 6
  Synthetic construct

SEQ ID NO: 25 - protein, 101 aa, Artificial Sequence; identical to SEQ ID NO: 7
  Synthetic construct

SEQ ID NO: 26 - protein, 406 aa, Artificial Sequence; identical to SEQ ID NO: 8
  Synthetic construct

SEQ ID NO: 27 - protein, 183 aa, Artificial Sequence; identical to SEQ ID NO: 9
  Synthetic construct

SEQ ID NO: 28 - protein, 44 aa, Artificial Sequence; identical to SEQ ID NO: 10
  Synthetic construct

SEQ ID NO: 29 - protein, 173 aa, Artificial Sequence; identical to SEQ ID NO: 11
  Synthetic construct

SEQ ID NO: 30 - protein, 204 aa, Artificial Sequence; identical to SEQ ID NO: 12
  Synthetic construct

SEQ ID NO: 31 - protein, 93 aa, Artificial Sequence; identical to SEQ ID NO: 21
  Synthetic construct